European Patent Specification EP 4 121 512 B1, published August 21, 2024. Title: Heart tissue model. Applicant: IMBA - INSTITUT FÜR MOLEKULARE BIOTECHNOLOGIE GMBH. The sequence listing filed with the application follows.

SEQUENCE LISTING (9 sequences)

SEQ ID NO: 1 - DNA, 20 bp, Artificial Sequence
  sgRNA
gagcattaacagcgcattcg

SEQ ID NO: 2 - DNA, 20 bp, Artificial Sequence
  sgRNA
gacgcacacttggccggtga

SEQ ID NO: 3 - DNA, 20 bp, Artificial Sequence
  sgRNA
acttggccggtgaaggcgcg

SEQ ID NO: 4 - DNA, 24 bp, Artificial Sequence
  primer
caccgagcattaacagcgcattcg

SEQ ID NO: 5 - DNA, 25 bp, Artificial Sequence
  primer
aaaccgaatgcgctgttaatgctcc

SEQ ID NO: 6 - DNA, 25 bp, Artificial Sequence
  primer
caccggacgcacacttggccggtga

SEQ ID NO: 7 - DNA, 25 bp, Artificial Sequence
  primer
aaactcaccggccaagtgtgcgtcc

SEQ ID NO: 8 - DNA, 25 bp, Artificial Sequence
  primer
caccgacttggccggtgaaggcgcg

SEQ ID NO: 9 - DNA, 24 bp, Artificial Sequence
  primer
aaaccgcgccttcaccggccaagt